European Patent Application EP 4 722 324 A1, published April 8, 2026. Title: Cleaning composition comprising a mannanase. Applicant: BASF SE. The sequence listing filed with the application follows.

SEQUENCE LISTING (15 sequences)

SEQ ID NO: 1 - protein, 269 aa, Bacillus lentus
  REGION 1..269: note = wildtype
AQSVPWGISRVQAPAAHNRGLTGSGVKVAVLDTGISTHPDLNIRGGASFVPGEPSTQDGNGHGTHVAGTIAALNNSIGVLGVAPSAELYAVKVLGADGRGAISSIAQGLEWAGNNGMHVANLSLGSPSPSATLEQAVNSATSRGVLVVAASGNSGASSISYPARYANAMAVGATDQNNNRASFSQYGAGLDIVAPGVNVQSTYPGSTYASLNGTSMATPHVAGAAALVKQKNPSWSNVQIRNHLKNTATSLGSTNLYGSGLVNAEAATR

SEQ ID NO: 2 - protein, 275 aa, Bacillus amyloliquefaciens [sequence omitted]

SEQ ID NO: 3 - protein, 269 aa, synthetic construct
AQSVPWGISRVQAPAAHNRGLTGSGVKVAVLDTGISTHPDLNIRGGASFVPGEPSTQDGNGHGTHVAGTIAALNNSIGVLGVAPSAELYAVKVLGADGEGAISSIAQGLEWAGNNGMHVANLSLGSPSPSATLEQAVNSATSRGVLVVAASGNSGASSISYPARYANAMAVGATDQNNNRASFSQYGAGLDIVAPGVNVQSTYPGSTYASLNGTSMATPHVAGAAALVKQKNPSWSNVQIRNHLKNTATSLGSTNLYGSGLVNAEAATR

SEQ ID NO: 4 - protein, 7 aa, synthetic construct
  REGION 1..7: note = loop sequence
ADGEGAI

SEQ ID NO: 5 - protein, 7 aa, synthetic construct
  REGION 1..7: note = loop sequence
ADGDGAI

SEQ ID NO: 6 - protein, 7 aa, synthetic construct
  REGION 1..7: note = loop sequence
ADGDGSV

SEQ ID NO: 7 - protein, 7 aa, synthetic construct
  REGION 1..7: note = loop sequence
ADGEGSV

SEQ ID NO: 8 - protein, 8 aa, synthetic construct
  REGION 1..8: note = loop sequence
AADGEGSV

SEQ ID NO: 9 - protein, 8 aa, synthetic construct
  REGION 1..8: note = loop sequence
ASEGEGSV

SEQ ID NO: 10 - protein, 4 aa, synthetic construct
AAPF

SEQ ID NO: 11 - protein, 460 aa, synthetic construct
ATGFYVNGNTLYDATGSPFVMRGINHAHSWFKDDSSTAIPAIAKTGANTIRIVLSDGSQYTKDDINTVKSLISLAEKNNLIAILEVHDATGNDAVSSLNDAVSYWISIKEALIGKEDRVLINIANEWYGTWDGASWASGYKQAIPKLRDAGLSHTLIVDSAGWGQYPESIHQYGKDVFNADPLKNTMFSIHMYEYAGGDASTIKSNIDGVLNQDLALIIGEFGHKHTNGDVDEETIMSYSQQKNVGWLAWSWKGNGPEWSYLDLSNDWAGDNLTSWGNTIVNGANGLKATSKISPVFDGGDHPGGSGGTENTLYNFETETQSWSGGNVMAGPWSTNEWASKDNYSLKADVQLNNNSQHYLSLTQNQNFSGKSQLKATVKHADWGNLGNGINAQLYVKTGSDWKWFDGESVEINSSNGTILTLDLSSISDLNDIKEIGVQFMGSSKSSGQTAVYVDNVTIQ

SEQ ID NO: 12 - protein, 460 aa, synthetic construct
ATGFYVNGNTLYDATGSPFVMRGINHAHSWFKDDSSTAIPAIAKTGANTIRIVLSDGSVYTKDDIDTVKSLISLAEKNNLIAILEVHDHTGNDAVSSLNDAVSYWISIKEALIGKEDRVLINIANEWYGTWDGASWASGYKQAIPKLRDAGLSHTLIVDSAGWGQYPESIHQYGKDVFNADPLKNTMFSIHMYEYAGGDASTIKSNIDGVLNQDLALIIGEFGHKHTNGDVDEQTIMSYSQQKNVGWLAWSWKGNGPEMSYLDLSNDWAGDNLTSWGNTIVYGANGLKATSKISPVFDGGDHPGGSGGTENTLYNFENGTQGWSGGNVMAGPWSTNEWASKDNYSLKADVQLNNNSQHYLSLTQNQNFSGKSQLKATVKHADWGNLGNGINAQLYVKTGSDWKWFDGESVEINSSNGTILTLDLSSISDLNDIKEIGVQFMGSSKSSGQTAVYVDNVTIQ

SEQ ID NO: 13 - protein, 298 aa, synthetic construct
MATGFYVSGNKLYDSTGKEFVMRGVNHGHTWFKNDLNEAIPAIAKTGANTVRIVLSNGVQYTRDDLDAVKNIINVVNQNKMIAVLEVHDATGKDDYDSLDAAINYWISIKEALIGKEDRVIVNIANEWMGTWNGSAWADGYKKAIPKLRNAGIKNTLIVDAAGWGQYPQSIVDYGQSVFAADSLKNTVFSIHMYEYAGKDAATVKANMENVLNKGLALIIGEFGCYHVNGDVDELAIMRYGQELGVGWLAWSWYGNSDGLRYLDMATGPNGSLTSFGNTVVNDTYGIKNTSQKAGIFQ

SEQ ID NO: 14 - protein, 483 aa, synthetic construct
HHNGTNGTMMQYFEWYLPNDGNHWNRLRSDASNLKDKGITAVWIPPAWKGASQNDVGYGAYDLYDLGEFNQKGTVRTKYGTRNQLQAAVTALKSNGIQVYGDVVMNHKGGADATEWVRAVEVNPSNRNQEVSGDYTIEAWTKFDFPGRGNTHSNFKWRWYHFDGVDWDQSRQLQNRIYKFRGKGWDWEVDTENGNYDYLMYADIDMDHPEVVNELRNWGVWYTNTLGLDGFRIDAVKHIKYSFTRDWLTHVRNTTGKNMFAVAEFWKNDIGAIENYLSKTNWNHSVFDVPLHYNLYNASRSGGNYDMRQIFNGTVVQRHPTHAVTFVDNHDSQPEEALESFVEEWFKPLAYALTLTRDQGYPSVFYGDYYGIPTHGVPAMKSKIDPILEARQKYAYGTQRDYLDHPDVIGWTREGDGVHADSGLATLMSDGPGGSKWMEVGKNNAGEVWYDITGNQTNTVTINKDGWGQFHVSGGSVSIYVQQ

SEQ ID NO: 15 - protein, 485 aa, synthetic construct
HHNGTNGTMMQYFEWYLPNDGNHWNRLRSDASNLKDKGITAVWIPPAWKGASQNDVGYGAYDLYDLGEFNQKGTVRTKYGTRNQLQAAVTALKSNGIQVYGDVVMNHKGGADATEWVRAVEVNPSNRNQEVSGDYTIEAWTKFDFPGRGNTHSNFKWRWYHFDGVDWDQSRQLQNRIYKFRGDGKGWDWEVDTENGNYDYLMYADIDMDHPEVVNELRNWGVWYTNTLGLDGFRIDAVKHIKYSFTRDWLTHVRNTTGKNMFAVAEFWKNDIGAIENYLSKTNWNHSVFDVPLHYNLYNASRSGGNYDMRQIFNGTVVQRHPTHAVTFVDNHDSQPEEALESFVEEWFKPLAYALTLTRDQGYPSVFYGDYYGIPTHGVPAMKSKIDPILEARQKYAYGKQNDYLDHHNMIGWTREGNTAHPNSGLATIMSDGPGGNKWMYVGRNKAGQVWRDITGNRSGTVTINADGWGNFSVNGGSVSIWVNN